European Patent Specification EP 4 083 203 B1, published August 7, 2024. Title: COMPOSITIONS AND METHODS FOR REDUCING OCULAR NEOVASCULARIZATION. Applicant: ADVERUM BIOTECHNOLOGIES, INC. Application PCT/US2017/038012. The sequence listing filed with the application follows.

SEQUENCE LISTING (13 sequences)

SEQ ID NO: 1 - protein, 7 aa, Artificial Sequence
  Description of Artificial Sequence: Synthetic peptide
LGETTRP

SEQ ID NO: 2 - protein, 7 aa, Artificial Sequence
  Description of Artificial Sequence: Synthetic peptide
NETITRP

SEQ ID NO: 3 - protein, 7 aa, Artificial Sequence
  Description of Artificial Sequence: Synthetic peptide
KAGQANN

SEQ ID NO: 4 - protein, 7 aa, Artificial Sequence
  Description of Artificial Sequence: Synthetic peptide
KDPKTTN

SEQ ID NO: 5 - protein, 7 aa, Artificial Sequence
  Description of Artificial Sequence: Synthetic peptide
KDTDTTR

SEQ ID NO: 6 - protein, 7 aa, Artificial Sequence
  Description of Artificial Sequence: Synthetic peptide
RAGGSVG

SEQ ID NO: 7 - protein, 7 aa, Artificial Sequence
  Description of Artificial Sequence: Synthetic peptide
AVDTTKF

SEQ ID NO: 8 - protein, 7 aa, Artificial Sequence
  Description of Artificial Sequence: Synthetic peptide
STGKVPN

SEQ ID NO: 9 - protein, 214 aa, Artificial Sequence
  Description of Artificial Sequence: Synthetic polypeptide
DIQLTQSPSSLSASVGDRVTITCSASQDISNYLNWYQQKPGKAPKVLIYFTSSLHSGVPSRFSGSGSGTDFTLTISSLQPEDFATYYCQQYSTVPWTFGQGTKVEIKRTVAAPSVFIFPPSDEQLKSGTASVVCLLNNFYPREAKVQWKVDNALQSGNSQESVTEQDSKDSTYSLSSTLTLSKADYEKHKVYACEVTHQGLSSPVTKSFNRGEC

SEQ ID NO: 10 - protein, 231 aa, Artificial Sequence
  Description of Artificial Sequence: Synthetic polypeptide
EVQLVESGGGLVQPGGSLRLSCAASGYDFTHYGMNWVRQAPGKGLEWVGWINTYTGEPTYAADFKRRFTFSLDTSKSTAYLQMNSLRAEDTAVYYCAKYPYYYGTSHWYFDVWGQGTLVTVSSASTKGPSVFPLAPSSKSTSGGTAALGCLVKDYFPEPVTVSWNSGALTSGVHTFPAVLQSSGLYSLSSVVTVPSSSLGTQTYICNVNHKPSNTKVDKKVEPKSCDKTHL

SEQ ID NO: 11 - protein, 214 aa, Artificial Sequence
  Description of Artificial Sequence: Synthetic polypeptide
DIQMTQSPSSLSASVGDRVTITCSASQDISNYLNWYQQKPGKAPKVLIYFTSSLHSGVPSRFSGSGSGTDFTLTISSLQPEDFATYYCQQYSTVPWTFGQGTKVEIKRTVAAPSVFIFPPSDEQLKSGTASVVCLLNNFYPREAKVQWKVDNALQSGNSQESVTEQDSKDSTYSLSSTLTLSKADYEKHKVYACEVTHQGLSSPVTKSFNRGEC

SEQ ID NO: 12 - protein, 453 aa, Artificial Sequence
  Description of Artificial Sequence: Synthetic polypeptide
EVQLVESGGGLVQPGGSLRLSCAASGYTFTNYGMNWVRQAPGKGLEWVGWINTYTGEPTYAADFKRRFTFSLDTSKSTAYLQMNSLRAEDTAVYYCAKYPHYYGSSHWYFDVWGQGTLVTVSSASTKGPSVFPLAPSSKSTSGGTAALGCLVKDYFPEPVTVSWNSGALTSGVHTFPAVLQSSGLYSLSSVVTVPSSSLGTQTYICNVNHKPSNTKVDKKVEPKSCDKTHTCPPCPAPELLGGPSVFLFPPKPKDTLMISRTPEVTCVVVDVSHEDPEVKFNWYVDGVEVHNAKTKPREEQYNSTYRVVSVLTVLHQDWLNGKEYKCKVSNKALPAPIEKTISKAKGQPREPQVYTLPPSREEMTKNQVSLTCLVKGFYPSDIAVEWESNGQPENNYKTTPPVLDSDGSFFLYSKLTVDKSRWQQGNVFSCSVMHEALHNHYTQKSLSLSPGK

SEQ ID NO: 13 - DNA, 2064 bp, Homo sapiens
atggtcagctactgggacaccggggtcctgctgtgcgcgctgctcagctgtctgcttctcacaggatctagttcaggttcaaaattaaaagatcctgaactgagtttaaaaggcacccagcacatcatgcaagcaggccagacactgcatctccaatgcaggggggaagcagcccataaatggtctttgcctgaaatggtgagtaaggaaagcgaaaggctgagcataactaaatctgcctgtggaagaaatggcaaacaattctgcagtactttaaccttgaacacagctcaagcaaaccacactggcttctacagctgcaaatatctagctgtacctacttcaaagaagaaggaaacagaatctgcaatctatatatttattagtgatacaggtagacctttcgtagagatgtacagtgaaatccccgaaattatacacatgactgaaggaagggagctcgtcattccctgccgggttacgtcacctaacatcactgttactttaaaaaagtttccacttgacactttgatccctgatggaaaacgcataatctgggacagtagaaagggcttcatcatatcaaatgcaacgtacaaagaaatagggcttctgacctgtgaagcaacagtcaatgggcatttgtataagacaaactatctcacacatcgacaaaccaatacaatcatagatgtccaaataagcacaccacgcccagtcaaattacttagaggccatactcttgtcctcaattgtactgctaccactcccttgaacacgagagttcaaatgacctggagttaccctgatgaaaaaaataagagagcttccgtaaggcgacgaattgaccaaagcaattcccatgccaacatattctacagtgttcttactattgacaaaatgcagaacaaagacaaaggactttatacttgtcgtgtaaggagtggaccatcattcaaatctgttaacacctcagtgcatatatatgataaagcattcatcactgtgaaacatcgaaaacagcaggtgcttgaaaccgtagctggcaagcggtcttaccggctctctatgaaagtgaaggcatttccctcgccggaagttgtatggttaaaagatgggttacctgcgactgagaaatctgctcgctatttgactcgtggctactcgttaattatcaaggacgtaactgaagaggatgcagggaattatacaatcttgctgagcataaaacagtcaaatgtgtttaaaaacctcactgccactctaattgtcaatgtgaaaccccagatttacgaaaaggccgtgtcatcgtttccagacccggctctctacccactgggcagcagacaaatcctgacttgtaccgcatatggtatccctcaacctacaatcaagtggttctggcacccctgtaaccataatcattccgaagcaaggtgtgacttttgttccaataatgaagagtcctttatcctggatgctgacagcaacatgggaaacagaattgagagcatcactcagcgcatggcaataatagaaggaaagaataagatggctagcaccttggttgtggctgactctagaatttctggaatctacatttgcatagcttccaataaagttgggactgtgggaagaaacataagcttttatatcacagatgtgccaaatgggtttcatgttaacttggaaaaaatgccgacggaaggagaggacctgaaactgtcttgcacagttaacaagttcttatacagagacgttacttggattttactgcggacagttaataacagaacaatgcactacagtattagcaagcaaaaaatggccatcactaaggagcactccatcactcttaatcttaccatcatgaatgtttccctgcaagattcaggcacctatgcctgcagagccaggaatgtatacacaggggaagaaatcctccagaagaaagaaattacaatcagaggtgagcactgcaacaaaaaggctgttttctctcggatctccaaatttaaaagcacaaggaatgattgtaccacacaaagtaatgtaaaacattaa